European Patent Application EP 4 624 572 A1, published October 1, 2025. Title: Polypeptides having protease activity for use in detergent compositions. Applicant: BASF SE. The sequence listing filed with the application follows.

SEQUENCE LISTING (57 sequences)

SEQ ID NO: 1 - protein, 269 aa, synthetic construct
AQSVPWGIARVQAPAAHQRGVTGKDVKVAVLDTGISWHPDLKIRGGASFVPGEPDTQDGNGHGTHVAGTIAALNNNIGVLGVAPSAELYAVKVLGADGEGSISSIAKGLEWAGNNGMHVANLSLGSPSPSATLEQAVNSATNRGVLVVAASGNSGASHISYPARYANAMAVGATDKDNNRASFSQYGEGLDIVAPGVDVQSTYIGPTYASLSGTSMATPHVSGAAALVKQKNPSWSNVQIRQHLKNTATSLGSDFLYGSGLVNADAATR

SEQ ID NO: 2 - protein, 269 aa, synthetic construct
AQSVPWGIARVQAPAAHQRGVTGKDVKVAVLDTGISKHPDLKIRGGASFVPGEPDTQDGNGHGTHVAGTIAALNNNIGVLGVAPSAELYAVKVLGADGEGSISSIAKGLEWAGNNGMHVANLSLGSPSPSATLEQAVNSATNRGVLVVAASGNSGASHISYPARYANAMAVGATDKDNNRASFSQYGEGLDIVAPGVDVQSTYIGPTYASLSGTSMATPHVSGAAALVKQKNPSWSNVQIRQHLKNTATSLGSDNLYGSGLVNADAATR

SEQ ID NO: 3 - protein, 269 aa, synthetic construct
AQSVPWGIARVQAPAAHQRGVTGKDVKVAVLDTGISKHPDLKIRGGASFVPGEPDTQDGNGHGTHVAGTIAALNNNIGVLGVAPSAELYAVKVLGADGEGSISSIAKGLEWAGNNGMHVANLSLGSPSPSATLEQAVNSATNRGVLVVAASGNSGASHISYPARYANAMAVGATDKDNNRASFSQYGEGLDIVAPGVDVQSTYIGPTYASLSGTSMATPHVSGAAALVKQKNPSWSNVQIRQHLKNTATSLGSDFLYGSGLVNADAATR

SEQ ID NO: 4 - protein, 269 aa, synthetic construct
AQSVPWGIARVQAPAAHQRGVTGKDVKVAVLDTGISKHPDLKIRGGASFVPGEPDTQDGNGHGTHVAGTIAALNNNIGVLGVAPSAELYAVKVLGADGEGSISSIAKGLEWAGNNGMHVANLSLGSPSPSATLEQAVNSATNRGVLVVAASGNSGASHISYPARYANAMAVGATDKDNNRASFSQYGEGLDIVAPGVDVQSTYIGPTYASLSGTSMATPHVSGAAALVKQKNPSWSNVQIRQHLKNTATSLGDDFLYGSGLVNADAATR

SEQ ID NO: 5 - protein, 269 aa, synthetic construct
AQSVPWGISRVQAPAAHQRGVTGKDVKVAVLDTGISKHPDLNIRGGASFVPGEPDTQDGNGHGTHVAGTIAALNNNIGVLGVAPSAELYAVKVLGADGEGSISSIAKGLEWAGNNGMHVANLSLGSPSPSATLEQAVNSATNRGVLVVAASGNSGASHISYPARYANAMAVGATDKDNNRASFSQYGEGLDIVAPGVDVQSTYIGPTYASLSGTSMATPHVSGAAALVKQKNPSWSNVQIRQHLKNTATSLGSDFLYGSGLVNADAATR

SEQ ID NO: 6 - protein, 269 aa, synthetic construct
AQSVPWGISRVQAPAAHQRGVTGKGVKVAVLDTGISWHPDLNIRGGASFVPGEPDTQDGNGHGTHVAGTIAALNNNIGVLGVAPSAELYAVKVLGADGEGSISSIAKGLEWAGNNGMHVANLSLGSPSPSATLEQAVNSATNRGVLVVAASGNSGASHISYPARYANAMAVGATDKDNNRASFSQYGEGLDIVAPGVDVQSTYIGPTYASLSGTSMATPHVSGAAALVKQKNPSWSNVQIRQHLKNTATSLGSDFLYGSGLVNADAATR

SEQ ID NO: 7 - protein, 269 aa, synthetic construct
AQSVPWGIARVQAPAAHQRGVTGKDVKVAVLDTGISKHPDLNIRGGASFVPGEPDTQDGNGHGTHVAGTIAALNNNIGVLGVAPSAELYAVKVLGADGEGSISSIAKGLEWAGNNGMHVANLSLGSPSPSATLEQAVNSATNRGVLVVAASGNSGASHISYPARYANAMAVGATDKDNNRASFSQYGAGLDIVAPGVDVQSTYIGPTYASLSGTSMATPHVSGAAALVKQKNPSWSNVQIRQHLKNTATSLGDDFLYGSGLVNADAATR

SEQ ID NO: 8 - protein, 269 aa, synthetic construct
AQSVPWGIARVQAPAAHQRGVTGKGVKVAVLDTGISKHPDLNIRGGASFVPGEPDTQDGNGHGTHVAGTIAALNNNIGVLGVAPSAELYAVKVLGADGEGSISSIAKGLEWAGNNGMHVANLSLGSPSPSATLEQAVNSATNRGVLVVAASGNSGASHISYPARYANAMAVGATDKDNNRASFSQYGEGLDIVAPGVDVQSTYIGPTYASLSGTSMATPHVSGAAALVKQKNPSWSNVQIRQHLKNTATSLGSDFLYGSGLVNADAATR

SEQ ID NO: 9 - protein, 269 aa, synthetic construct
AQSVPWGIARVQAPAAHQRGVTGKGVKVAVLDTGISKHPDLNIRGGASFVPGEPDTQDGNGHGTHVAGTIAALNNNIGVLGVAPSAELYAVKVLGADGEGSISSIAKGLEWAGNNGMHVANLSLGSPSPSATLEQAVNSATNRGVLVVAASGNSGASHISYPARYANAMAVGATDKDNNRASFSQYGEGLDIVAPGVDVQSTYIGPTYASLSGTSMATPHVSGAAALVKQKNPSWSNVQIRQHLKNTATSLGDDFLYGSGLVNADAATR

SEQ ID NO: 10 - protein, 269 aa, synthetic construct
AQSVPWGISRVQAPAAHQRGVTGKGVKVAVLDTGISKHPDLNIRGGASFVPGEPDTQDGNGHGTHVAGTIAALNNNIGVLGVAPSAELYAVKVLGADGEGSISSIAKGLEWAGNNGMHVANLSLGSPSPSATLEQAVNSATNRGVLVVAASGNSGASHISYPARYANAMAVGATDKDNNRASFSQYGAGLDIVAPGVDVQSTYIGPTYASLSGTSMATPHVSGAAALVKQKNPSWSNVQIRQHLKNTATSLGDDFLYGSGLVNADAATR

SEQ ID NO: 11 - protein, 269 aa, synthetic construct
AQSVPWGISRVQAPAAHQRGVTGKDVKVAVLDTGISKHPDLKIRGGASFVPGEPDTQDGNGHGTHVAGTIAALNNNIGVLGVAPSAELYAVKVLGADGEGSISSIAKGLEWAGNNGMHVANLSLGSPSPSATLEQAVNSATNRGVLVVAASGNSGASHISYPARYANAMAVGATDKDNNRASFSQYGEGLDIVAPGVDVQSTYIGSTYASLSGTSMATPHVSGAAALVKQKNPSWSNVQIRQHLKNTATSLGSDFLYGSGLVNADAATR

SEQ ID NO: 12 - protein, 269 aa, synthetic construct
AQSVPWGIARVQAPAAHQRGVTGKDVKVAVLDTGISKHPDLKIRGGASFVPGEPDTQDGNGHGTHVAGTIAALNNNIGVLGVAPSAELYAVKVLGADGEGSISSIAKGLEWAGNNGMHVANLSLGSPSPSATLEQAVNSATNRGVLVVAASGNSGASHISYPARYANAMAVGATDKDNNRASFSQYGEGLDIVAPGVDVQSTYIGSTYASLSGTSMATPHVSGAAALVKQKNPSWSNVQIRQHLKNTATSLGSDFLYGSGLVNADAATR

SEQ ID NO: 13 - protein, 269 aa, synthetic construct
AQSVPWGIARVQAPAAHQRGVTGKDVKVAVLDTGISKHPDLKIRGGASFVPGEPDTQDGNGHGTHVAGTIAALNNNIGVLGVAPSAELYAVKVLGADGEGSISSIAKGLEWAGNNGMHVANLSLGSPSPSATLEQAVNSATNRGVLVVAASGNSGASHISYPARYANAMAVGATDKDNNRASFSQYGAGLDIVAPGVDVQSTYIGSTYASLSGTSMATPHVSGAAALVKQKNPSWSNVQIRQHLKNTATSLGSDFLYGSGLVNADAATR

SEQ ID NO: 14 - protein, 269 aa, synthetic construct
AQSVPWGIARVQAPAAHQRGVTGKGVKVAVLDTGISKHPDLKIRGGASFVPGEPDTQDGNGHGTHVAGTIAALNNNIGVLGVAPSAELYAVKVLGADGEGSISSIAKGLEWAGNNGMHVANLSLGSPSPSATLEQAVNSATNRGVLVVAASGNSGASHISYPARYANAMAVGATDKDNNRASFSQYGEGLDIVAPGVDVQSTYIGSTYASLSGTSMATPHVSGAAALVKQKNPSWSNVQIRQHLKNTATSLGSDFLYGSGLVNADAATR

SEQ ID NO: 15 - protein, 269 aa, synthetic construct
AQSVPWGIARVQAPAAHQRGVTGKGVKVAVLDTGISKHPDLNIRGGASFVPGEPDTQDGNGHGTHVAGTIAALNNNIGVLGVAPSAELYAVKVLGADGEGAISSIAKGLEWAGNNGMHVANLSLGSPSPSATLEQAVNSATNRGVLVVAASGNSGASHISYPARYANAMAVGATDKDNNRASFSQYGAGLDIVAPGVDVQSTYIGSTYASLSGTSMATPHVSGAAALVKQKNPSWSNVQIRQHLKNTATSLGSDNLYGSGLVNADAATR

SEQ ID NO: 16 - protein, 269 aa, synthetic construct
AQSVPWGISRVQAPAAHQRGVTGKDVKVAVLDTGISKHPDLRIRGGASFVPGEPDTQDGNGHGTHVAGTIAALNNNIGVLGVAPSAELYAVKVLGADGEGSISSIAKGLEWAGNNGMHVANLSLGSPSPSATLEQAVNSATNRGVLVVAASGNSGASHISYPARYANAMAVGATDKDNNRASFSQYGEGLDIVAPGVDVQSTYIGPTYASLSGTSMATPHVSGAAALVKQKNPSWSNVQIRQHLKNTATSLGSTFLYGSGLVNAEAATR

SEQ ID NO: 17 - protein, 269 aa, synthetic construct
AQSVPWGISRVQAPAAHQRGVTGKDVKVAVLDTGISKHPDLRIRGGASFVPGEPDTQDGNGHGTHVAGTIAALNNNIGVLGVAPSAELYAVKVLGADGEGAISSIAKGLEWAGNNGMHVANLSLGSPSPSATLEQAVNSATNRGVLVVAASGNSGASHISYPARYANAMAVGATDKDNNRASFSQYGEGLDIVAPGVDVQSTYIGPTYASLSGTSMATPHVSGAAALVKQKNPSWSNVQIRQHLKNTATSLGSTNLYGSGLVNAEAATR

SEQ ID NO: 18 - protein, 269 aa, synthetic construct
AQSVPWGIARVQAPAAHQRGVTGKDVKVAVLDTGISKHPDLRIRGGASFVPGEPDTQDGNGHGTHVAGTIAALNNNIGVLGVAPSAELYAVKVLGADGEGSISSIAKGLEWAGNNGMHVANLSLGSPSPSATLEQAVNSATNRGVLVVAASGNSGASHISYPARYANAMAVGATDKDNNRASFSQYGEGLDIVAPGVDVQSTYIGPTYASLSGTSMATPHVSGAAALVKQKNPSWSNVQIRQHLKNTATSLGSTFLYGSGLVNADAATR

SEQ ID NO: 19 - protein, 269 aa, synthetic construct
AQSVPWGISRVQAPAAHQRGVTGKDVKVAVLDTGISKHPDLKIRGGASFVPGEPDTQDGNGHGTHVAGTIAALNNNIGVLGVAPSAELYAVKVLGADGEGAISSIAKGLEWAGNNGMHVANLSLGSPSPSATLEQAVNSATNRGVLVVAASGNSGASHISYPARYANAMAVGATDKDNNRASFSQYGEGLDIVAPGVDVQSTYIGPTYASLSGTSMATPHVSGAAALVKQKNPSWSNVQIRQHLKNTATSLGDTFLYGSGLVNAEAATR

SEQ ID NO: 20 - protein, 269 aa, synthetic construct
AQSVPWGIARVQAPAAHQRGVTGKDVKVAVLDTGISWHPDLKIRGGASFVPGEPDTQDGNGHGTHVAGTIAALNNNIGVLGVAPSAELYAVKVLGADGEGSISSIAKGLEWAGNNGMHVANLSLGSPSPSATLEQAVNSATNRGVLVVAASGNSGASHISYPARYANAMAVGATDKDNNRASFSQYGAGLDIVAPGVDVQSTYIGPTYASLSGTSMATPHVSGAAALVKQKNPSWSNVQIRQHLKNTATSLGDTFLYGSGLVNADAATR

SEQ ID NO: 21 - protein, 269 aa, synthetic construct
AQSVPWGIARVQAPAAHQRGVTGKDVKVAVLDTGISKHPDLKIRGGASFVPGEPDTQDGNGHGTHVAGTIAALNNNIGVLGVAPSAELYAVKVLGADGEGSISSIAKGLEWAGNNGMHVANLSLGSPSPSATLEQAVNSATNRGVLVVAASGNSGASHISYPARYANAMAVGATDKDNNRASFSQYGEGLDIVAPGVDVQSTYIGPTYASLSGTSMATPHVSGAAALVKQKNPSWSNVQIRQHLKNTATSLGDTNLYGSGLVNADAATR

SEQ ID NO: 22 - protein, 269 aa, synthetic construct
AQSVPWGIARVQAPAAHQRGVTGKDVKVAVLDTGISKHPDLKIRGGASFVPGEPDTQDGNGHGTHVAGTIAALNNNIGVLGVAPSAELYAVKVLGADGEGSISSIAKGLEWAGNNGMHVANLSLGSPSPSATLEQAVNSATNRGVLVVAASGNSGASHISYPARYANAMAVGATDKDNNRASFSQYGEGLDIVAPGVDVQSTYIGPTYASLSGTSMATPHVSGAAALVKQKNPSWSNVQIRQHLKNTATSLGDTFLYGSGLVNAEAATR

SEQ ID NO: 23 - protein, 269 aa, synthetic construct
AQSVPWGIARVQAPAAHQRGVTGKDVKVAVLDTGISKHPDLKIRGGASFVPGEPDTQDGNGHGTHVAGTIAALNNNIGVLGVAPSAELYAVKVLGADGEGSISSIAKGLEWAGNNGMHVANLSLGSPSPSATLEQAVNSATNRGVLVVAASGNSGASHISYPARYANAMAVGATDKDNNRASFSQYGAGLDIVAPGVDVQSTYIGPTYASLSGTSMATPHVSGAAALVKQKNPSWSNVQIRQHLKNTATSLGDTNLYGSGLVNADAATR

SEQ ID NO: 24 - protein, 269 aa, synthetic construct
AQSVPWGIARVQAPAAHQRGVTGKDVKVAVLDTGISKHPDLKIRGGASFVPGEPDTQDGNGHGTHVAGTIAALNNNIGVLGVAPSAELYAVKVLGADGEGSISSIAKGLEWAGNNGMHVANLSLGSPSPSATLEQAVNSATNRGVLVVAASGNSGASHISYPARYANAMAVGATDKDNNRASFSQYGAGLDIVAPGVDVQSTYIGPTYASLSGTSMATPHVSGAAALVKQKNPSWSNVQIRQHLKNTATSLGDTFLYGSGLVNADAATR

SEQ ID NO: 25 - protein, 269 aa, synthetic construct
AQSVPWGIARVQAPAAHQRGVTGKGVKVAVLDTGISKHPDLKIRGGASFVPGEPDTQDGNGHGTHVAGTIAALNNNIGVLGVAPSAELYAVKVLGADGEGSISSIAKGLEWAGNNGMHVANLSLGSPSPSATLEQAVNSATNRGVLVVAASGNSGASHISYPARYANAMAVGATDKDNNRASFSQYGEGLDIVAPGVDVQSTYIGPTYASLSGTSMATPHVSGAAALVKQKNPSWSNVQIRQHLKNTATSLGDTFLYGSGLVNAEAATR

SEQ ID NO: 26 - protein, 269 aa, synthetic construct
AQSVPWGIARVQAPAAHQRGVTGKGVKVAVLDTGISKHPDLKIRGGASFVPGEPDTQDGNGHGTHVAGTIAALNNNIGVLGVAPSAELYAVKVLGADGEGSISSIAKGLEWAGNNGMHVANLSLGSPSPSATLEQAVNSATNRGVLVVAASGNSGASHISYPARYANAMAVGATDKDNNRASFSQYGEGLDIVAPGVDVQSTYIGPTYASLSGTSMATPHVSGAAALVKQKNPSWSNVQIRQHLKNTATSLGDTFLYGSGLVNADAATR

SEQ ID NO: 27 - protein, 269 aa, synthetic construct
AQSVPWGIARVQAPAAHQRGVTGKGVKVAVLDTGISKHPDLKIRGGASFVPGEPDTQDGNGHGTHVAGTIAALNNNIGVLGVAPSAELYAVKVLGADGEGSISSIAKGLEWAGNNGMHVANLSLGSPSPSATLEQAVNSATNRGVLVVAASGNSGASHISYPARYANAMAVGATDKDNNRASFSQYGAGLDIVAPGVDVQSTYIGPTYASLSGTSMATPHVSGAAALVKQKNPSWSNVQIRQHLKNTATSLGDTFLYGSGLVNADAATR

SEQ ID NO: 28 - protein, 269 aa, synthetic construct
AQSVPWGISRVQAPAAHQRGVTGKGVKVAVLDTGISWHPDLNIRGGASFVPGEPDTKDGNGHGTHVAGTIAALNNNIGVLGVAPSAELYAVKVLGADGEGSISSIAKGLEWAGNNGMHVANLSLGSPSPSATLEQAVNSATNRGVLVVAASGNSGASHISYPARYANAMAVGATDKDNNRASFSQYGEGLDIVAPGVDVQSTYIGPTYASLSGTSMATPHVSGAAALVKQKNPSWSNVQIRQHLKNTATSLGSDFLYGSGLVNADAATR

SEQ ID NO: 29 - protein, 269 aa, synthetic construct
AQSVPWGIARVQAPAAHQRGVTGKDVKVAVLDTGISWHPDLNIRGGASFVPGEPDTKDGNGHGTHVAGTIAALNNNIGVLGVAPSAELYAVKVLGADGEGSISSIAKGLEWAGNNGMHVANLSLGSPSPSATLEQAVNSATNRGVLVVAASGNSGASHISYPARYANAMAVGATDKDNNRASFSQYGEGLDIVAPGVDVQSTYIGPTYASLSGTSMATPHVSGAAALVKQKNPSWSNVQIRQHLKNTATSLGSDFLYGSGLVNADAATR

SEQ ID NO: 30 - protein, 269 aa, synthetic construct
AQSVPWGIARVQAPAAHQRGVTGKDVKVAVLDTGISWHPDLNIRGGASFVPGEPDTKDGNGHGTHVAGTIAALNNNIGVLGVAPSAELYAVKVLGADGEGSISSIAKGLEWAGNNGMHVANLSLGSPSPSATLEQAVNSATNRGVLVVAASGNSGASHISYPARYANAMAVGATDKDNNRASFSQYGAGLDIVAPGVDVQSTYIGPTYASLSGTSMATPHVSGAAALVKQKNPSWSNVQIRQHLKNTATSLGDDFLYGSGLVNADAATR

SEQ ID NO: 31 - protein, 269 aa, synthetic construct
AQSVPWGIARVQAPAAHQRGVTGKDVKVAVLDTGISWHPDLNIRGGASFVPGEPDTKDGNGHGTHVAGTIAALNNNIGVLGVAPSAELYAVKVLGADGEGAISSIAKGLEWAGNNGMHVANLSLGSPSPSATLEQAVNSATNRGVLVVAASGNSGASHISYPARYANAMAVGATDKDNNRASFSQYGAGLDIVAPGVDVQSTYIGPTYASLSGTSMATPHVSGAAALVKQKNPSWSNVQIRQHLKNTATSLGSDNLYGSGLVNADAATR

SEQ ID NO: 32 - protein, 269 aa, synthetic construct
AQSVPWGIARVQAPAAHQRGVTGKDVKVAVLDTGISKHPDLNIRGGASFVPGEPDTKDGNGHGTHVAGTIAALNNNIGVLGVAPSAELYAVKVLGADGEGSISSIAKGLEWAGNNGMHVANLSLGSPSPSATLEQAVNSATNRGVLVVAASGNSGASHISYPARYANAMAVGATDKDNNRASFSQYGEGLDIVAPGVDVQSTYIGPTYASLSGTSMATPHVSGAAALVKQKNPSWSNVQIRQHLKNTATSLGSDNLYGSGLVNADAATR

SEQ ID NO: 33 - protein, 269 aa, synthetic construct
AQSVPWGIARVQAPAAHQRGVTGKDVKVAVLDTGISKHPDLNIRGGASFVPGEPDTKDGNGHGTHVAGTIAALNNNIGVLGVAPSAELYAVKVLGADGEGSISSIAKGLEWAGNNGMHVANLSLGSPSPSATLEQAVNSATNRGVLVVAASGNSGASHISYPARYANAMAVGATDKDNNRASFSQYGEGLDIVAPGVDVQSTYIGPTYASLSGTSMATPHVSGAAALVKQKNPSWSNVQIRQHLKNTATSLGSDFLYGSGLVNADAATR

SEQ ID NO: 34 - protein, 269 aa, synthetic construct
AQSVPWGIARVQAPAAHQRGVTGKDVKVAVLDTGISKHPDLNIRGGASFVPGEPDTKDGNGHGTHVAGTIAALNNNIGVLGVAPSAELYAVKVLGADGEGSISSIAKGLEWAGNNGMHVANLSLGSPSPSATLEQAVNSATNRGVLVVAASGNSGASHISYPARYANAMAVGATDKDNNRASFSQYGEGLDIVAPGVDVQSTYIGPTYASLSGTSMATPHVSGAAALVKQKNPSWSNVQIRQHLKNTATSLGDDNLYGSGLVNADAATR

SEQ ID NO: 35 - protein, 269 aa, synthetic construct
AQSVPWGIARVQAPAAHQRGVTGKDVKVAVLDTGISKHPDLNIRGGASFVPGEPDTKDGNGHGTHVAGTIAALNNNIGVLGVAPSAELYAVKVLGADGEGSISSIAKGLEWAGNNGMHVANLSLGSPSPSATLEQAVNSATNRGVLVVAASGNSGASHISYPARYANAMAVGATDKDNNRASFSQYGEGLDIVAPGVDVQSTYIGPTYASLSGTSMATPHVSGAAALVKQKNPSWSNVQIRQHLKNTATSLGDDFLYGSGLVNADAATR

SEQ ID NO: 36 - protein, 269 aa, synthetic construct
AQSVPWGIARVQAPAAHQRGVTGKDVKVAVLDTGISKHPDLNIRGGASFVPGEPDTKDGNGHGTHVAGTIAALNNNIGVLGVAPSAELYAVKVLGADGEGSISSIAKGLEWAGNNGMHVANLSLGSPSPSATLEQAVNSATNRGVLVVAASGNSGASHISYPARYANAMAVGATDKDNNRASFSQYGAGLDIVAPGVDVQSTYIGPTYASLSGTSMATPHVSGAAALVKQKNPSWSNVQIRQHLKNTATSLGDDFLYGSGLVNADAATR

SEQ ID NO: 37 - protein, 269 aa, synthetic construct
AQSVPWGIARVQAPAAHQRGVTGKDVKVAVLDTGISKHPDLNIRGGASFVPGEPDTKDGNGHGTHVAGTIAALNNNIGVLGVAPSAELYAVKVLGADGEGAISSIAKGLEWAGNNGMHVANLSLGSPSPSATLEQAVNSATNRGVLVVAASGNSGASHISYPARYANAMAVGATDKDNNRASFSQYGAGLDIVAPGVDVQSTYIGPTYASLSGTSMATPHVSGAAALVKQKNPSWSNVQIRQHLKNTATSLGDDNLYGSGLVNADAATR

SEQ ID NO: 38 - protein, 269 aa, synthetic construct
AQSVPWGIARVQAPAAHQRGVTGKGVKVAVLDTGISWHPDLNIRGGASFVPGEPDTKDGNGHGTHVAGTIAALNNNIGVLGVAPSAELYAVKVLGADGEGSISSIAKGLEWAGNNGMHVANLSLGSPSPSATLEQAVNSATNRGVLVVAASGNSGASHISYPARYANAMAVGATDKDNNRASFSQYGAGLDIVAPGVDVQSTYIGPTYASLSGTSMATPHVSGAAALVKQKNPSWSNVQIRQHLKNTATSLGDDFLYGSGLVNADAATR

SEQ ID NO: 39 - protein, 269 aa, synthetic construct
AQSVPWGISRVQAPAAHQRGVTGKGVKVAVLDTGISKHPDLNIRGGASFVPGEPDTKDGNGHGTHVAGTIAALNNNIGVLGVAPSAELYAVKVLGADGEGSISSIAKGLEWAGNNGMHVANLSLGSPSPSATLEQAVNSATNRGVLVVAASGNSGASHISYPARYANAMAVGATDKDNNRASFSQYGEGLDIVAPGVDVQSTYIGPTYASLSGTSMATPHVSGAAALVKQKNPSWSNVQIRQHLKNTATSLGSDNLYGSGLVNADAATR

SEQ ID NO: 40 - protein, 269 aa, synthetic construct
AQSVPWGISRVQAPAAHQRGVTGKGVKVAVLDTGISKHPDLNIRGGASFVPGEPDTKDGNGHGTHVAGTIAALNNNIGVLGVAPSAELYAVKVLGADGEGSISSIAKGLEWAGNNGMHVANLSLGSPSPSATLEQAVNSATNRGVLVVAASGNSGASHISYPARYANAMAVGATDKDNNRASFSQYGEGLDIVAPGVDVQSTYIGPTYASLSGTSMATPHVSGAAALVKQKNPSWSNVQIRQHLKNTATSLGSDFLYGSGLVNADAATR

SEQ ID NO: 41 - protein, 269 aa, synthetic construct
AQSVPWGISRVQAPAAHNRGLTGSGVKVAVLDTGISTHPDLNIRGGASFVPGEPSTQDGNGHGTHVAGTIAALNNSIGVLGVAPSAELYAVKVLGADGEGAISSIAQGLEWAGNNGMHVANLSLGSPSPSATLEQAVNSATSRGVLVVAASGNSGASSISYPARYANAMAVGATDQNNNRASFSQYGAGLDIVAPGVNVQSTYPGSTYASLNGTSMATPHVAGAAALVKQKNPSWSNVQIRNHLKNTATSLGSTNLYGSGLVNAEAATR

SEQ ID NO: 42 - protein, 275 aa, Bacillus amyloliquefaciens [sequence omitted]

SEQ ID NO: 43 - protein, 269 aa, synthetic construct
AQSVPWGISRVQAPAAHNRGLTGKGVKVAVLDTGISTHPDLKIRGGASFVPGEPDTQDGNGHGTHVAGTIAALNNNIGVLGVAPSAELYAVKVLGADGEGAISSIAKGLEWAGNNGMHVANLSLGSPSPSATLEQAVNSATNRGVLVVAASGNSGASSISYPARYANAMAVGATDKDNNRASFSQYGAGLDIVAPGVDVQSTYPGSTYASLNGTSMATPHVAGAAALVKQKNPSWSNVQIRQHLKNTATSLGSDNLYGSGLVNAEAATR

SEQ ID NO: 44 - protein, 4 aa, synthetic construct
AAPF

SEQ ID NO: 45 - protein, 269 aa, Bacillus lentus
AQSVPWGISRVQAPAAHNRGLTGSGVKVAVLDTGISTHPDLNIRGGASFVPGEPSTQDGNGHGTHVAGTIAALNNSIGVLGVAPSAELYAVKVLGADGRGAISSIAQGLEWAGNNGMHVANLSLGSPSPSATLEQAVNSATSRGVLVVAASGNSGASSISYPARYANAMAVGATDQNNNRASFSQYGAGLDIVAPGVNVQSTYPGSTYASLNGTSMATPHVAGAAALVKQKNPSWSNVQIRNHLKNTATSLGSTNLYGSGLVNAEAATR

SEQ ID NO: 46 - protein, 269 aa, synthetic construct
AQSVPWGISRVQAPAAHQRGVTGKGVKVAVLDTGISWHPDLKIRGGASFVPGEPDTQDGNGHGTHVAGTIAALNNNIGVLGVAPSAELYAVKVLGADGEGAISSIAKGLEWAGNNGMHVANLSLGSPSPSATLEQAVNSATNRGVLVVAASGNSGASHISYPARYANAMAVGATDKDNNRASFSQYGAGLDIVAPGVDVQSTYIGPTYASLSGTSMATPHVSGAAALVKQKNPSWSNVQIRQHLKNTATSLGSDNLYGSGLVNADAATR

SEQ ID NO: 47 - protein, 269 aa, synthetic construct
AQSVPWGISRVQAPAAHQRGVTGKDVKVAVLDTGISWHPDLKIRGGASFVPGEPDTQDGNGHGTHVAGTIAALNNNIGVLGVAPSAELYAVKVLGADGEGSISSIAKGLEWAGNNGMHVANLSLGSPSPSATLEQAVNSATNRGVLVVAASGNSGASHISYPARYANAMAVGATDKDNNRASFSQYGAGLDIVAPGVDVQSTYIGSTYASLSGTSMATPHVSGAAALVKQKNPSWSNVQIRQHLKNTATSLGSDNLYGSGLVNAEAATR

SEQ ID NO: 48 - protein, 269 aa, synthetic construct; identical to SEQ ID NO: 17

SEQ ID NO: 49 - protein, 269 aa, synthetic construct
AQSVPWGISRVQAPAAHQRGVTGKDVKVAVLDTGISKHPDLNIRGGASFVPGEPDTQDGNGHGTHVAGTIAALNNNIGVLGVAPSAELYAVKVLGADGEGSISSIAKGLEWAGNNGMHVANLSLGSPSPSATLEQAVNSATNRGVLVVAASGNSGASHISYPARYANAMAVGATDKDNNRASFSQYGAGLDIVAPGVDVQSTYIGPTYASLSGTSMATPHVSGAAALVKQKNPSWSNVQIRQHLKNTATSLGSDNLYGSGLVNADAATR

SEQ ID NO: 50 - protein, 269 aa, synthetic construct
AQSVPWGISRVQAPAAHQRGVTGKDVKVAVLDTGISWHPDLKIRGGASFVPGEPDTQDGNGHGTHVAGTIAALNNNIGVLGVAPSAELYAVKVLGADGEGSISSIAKGLEWAGNNGMHVANLSLGSPSPSATLEQAVNSATNRGVLVVAASGNSGASHISYPARYANAMAVGATDKDNNRASFSQYGEGLDIVAPGVDVQSTYIGSTYASLSGTSMATPHVSGAAALVKQKNPSWSNVQIRQHLKNTATSLGSDFLYGSGLVNADAATR

SEQ ID NO: 51 - protein, 269 aa, synthetic construct
AQSVPWGISRVQAPAAHQRGVTGKDVKVAVLDTGISKHPDLNIRGGASFVPGEPDTQDGNGHGTHVAGTIAALNNNIGVLGVAPSAELYAVKVLGADGEGSISSIAKGLEWAGNNGMHVANLSLGSPSPSATLEQAVNSATNRGVLVVAASGNSGASHISYPARYANAMAVGATDKDNNRASFSQYGAGLDIVAPGVDVQSTYIGPTYASLSGTSMATPHVSGAAALVKQKNPSWSNVQIRQHLKNTATSLGDDNLYGSGLVNADAATR

SEQ ID NO: 52 - protein, 269 aa, synthetic construct
AQSVPWGIARVQAPAAHQRGVTGKDVKVAVLDTGISWHPDLRIRGGASFVPGEPDTKDGNGHGTHVAGTIAALNNNIGVLGVAPSAELYAVKVLGADGEGAISSIAKGLEWAGNNGMHVANLSLGSPSPSATLEQAVNSATNRGVLVVAASGNSGASHISYPARYANAMAVGATDKDNNRASFSQYGAGLDIVAPGVDVQSTYIGPTYASLSGTSMATPHVSGAAALVKQKNPSWSNVQIRQHLKNTATSLGSDFLYGSGLVNADAATR

SEQ ID NO: 53 - protein, 269 aa, synthetic construct
AQSVPWGISRVQAPAAHQRGVTGKGVKVAVLDTGISWHPDLNIRGGASFVPGEPDTQDGNGHGTHVAGTIAALNNNIGVLGVAPSAELYAVKVLGADGEGSISSIAKGLEWAGNNGMHVANLSLGSPSPSATLEQAVNSATNRGVLVVAASGNSGASHISYPARYANAMAVGATDKDNNRASFSQYGEGLDIVAPGVDVQSTYIGSTYASLSGTSMATPHVSGAAALVKQKNPSWSNVQIRQHLKNTATSLGDDFLYGSGLVNADAATR

SEQ ID NO: 54 - protein, 269 aa, synthetic construct
AQSVPWGIARVQAPAAHQRGVTGKDVKVAVLDTGISWHPDLNIRGGASFVPGEPDTQDGNGHGTHVAGTIAALNNNIGVLGVAPSAELYAVKVLGADGEGSISSIAKGLEWAGNNGMHVANLSLGSPSPSATLEQAVNSATNRGVLVVAASGNSGASHISYPARYANAMAVGATDKDNNRASFSQYGEGLDIVAPGVDVQSTYIGPTYASLSGTSMATPHVSGAAALVKQKNPSWSNVQIRQHLKNTATSLGDDFLYGSGLVNAEAATR

SEQ ID NO: 55 - protein, 269 aa, synthetic construct
AQSVPWGIARVQAPAAHQRGVTGKDVKVAVLDTGISWHPDLNIRGGASFVPGEPDTQDGNGHGTHVAGTIAALNNNIGVLGVAPSAELYAVKVLGADGEGAISSIAKGLEWAGNNGMHVANLSLGSPSPSATLEQAVNSATNRGVLVVAASGNSGASHISYPARYANAMAVGATDKDNNRASFSQYGEGLDIVAPGVDVQSTYIGSTYASLSGTSMATPHVSGAAALVKQKNPSWSNVQIRQHLKNTATSLGSDFLYGSGLVNADAATR

SEQ ID NO: 56 - protein, 269 aa, synthetic construct
AQSVPWGIARVQAPAAHQRGVTGKGVKVAVLDTGISKHPDLRIRGGASFVPGEPDTKDGNGHGTHVAGTIAALNNNIGVLGVAPSAELYAVKVLGADGEGAISSIAKGLEWAGNNGMHVANLSLGSPSPSATLEQAVNSATNRGVLVVAASGNSGASHISYPARYANAMAVGATDKDNNRASFSQYGAGLDIVAPGVDVQSTYIGPTYASLSGTSMATPHVSGAAALVKQKNPSWSNVQIRQHLKNTATSLGDDFLYGSGLVNADAATR

SEQ ID NO: 57 - protein, 269 aa, synthetic construct
AQSVPWGIARVQAPAAHQRGVTGKGVKVAVLDTGISKHPDLNIRGGASFVPGEPDTQDGNGHGTHVAGTIAALNNNIGVLGVAPSAELYAVKVLGADGEGSISSIAKGLEWAGNNGMHVANLSLGSPSPSATLEQAVNSATNRGVLVVAASGNSGASHISYPARYANAMAVGATDKDNNRASFSQYGEGLDIVAPGVDVQSTYIGSTYASLSGTSMATPHVSGAAALVKQKNPSWSNVQIRQHLKNTATSLGSDFLYGSGLVNADAATR